European Patent Specification EP 3 515 506 B1, published September 13, 2023. Title: SILENCING OF DUX4 BY RECOMBINANT GENE EDITING COMPLEXES. Applicant: University of Massachusetts. Application Not Yet Assigned. The sequence listing filed with the application follows.

SEQUENCE LISTING (45 sequences)

SEQ ID NO: 1 - DNA, 22 bp, Artificial Sequence
  Synthetic polynucleotide
taccacagacagccaactgggg

SEQ ID NO: 2 - DNA, 22 bp, Artificial Sequence
  Synthetic polynucleotide
ttcacccagaacagtaactggg

SEQ ID NO: 3 - DNA, 22 bp, Artificial Sequence
  Synthetic polynucleotide
cacccgggcaaaagccgggagg

SEQ ID NO: 4 - DNA, 22 bp, Artificial Sequence
  Synthetic polynucleotide
ctggaagcacccctcagcgagg

SEQ ID NO: 5 - DNA, 22 bp, Artificial Sequence
  Synthetic polynucleotide
ctggaggagctttaggacgcgg

SEQ ID NO: 6 - DNA, 22 bp, Artificial Sequence
  Synthetic polynucleotide
ctcgctctggtcttctacgtgg

SEQ ID NO: 7 - DNA, 22 bp, Artificial Sequence
  Synthetic polynucleotide
ccgtccgtgaaattccggccgg

SEQ ID NO: 8 - DNA, 22 bp, Artificial Sequence
  Synthetic polynucleotide
tcggacagcaccctccccgcgg

SEQ ID NO: 9 - DNA, 22 bp, Artificial Sequence
  Synthetic polynucleotide
ctcccttgcacgtcagccgggg

SEQ ID NO: 10 - DNA, 22 bp, Artificial Sequence
  Synthetic polynucleotide
gaatttcacggaagaacaaggg

SEQ ID NO: 11 - DNA, 22 bp, Artificial Sequence
  Synthetic polynucleotide
atcttctataggatccacaggg

SEQ ID NO: 12 - DNA, 23 bp, Artificial Sequence
  Synthetic polynucleotide
gctctgctggaggagctttagga

SEQ ID NO: 13 - DNA, 20 bp, Artificial Sequence
  Synthetic polynucleotide
gcaggtctgcwggtacctgg

SEQ ID NO: 14 - DNA, 20 bp, Artificial Sequence
  Synthetic polynucleotide
tggaggccagggttcgtgaa

SEQ ID NO: 15 - DNA, 22 bp, Artificial Sequence
  Synthetic polynucleotide
attgttcctccgcttcttcagc

SEQ ID NO: 16 - DNA, 22 bp, Artificial Sequence
  Synthetic polynucleotide
tctacagagacgtaggctgtca

SEQ ID NO: 17 - DNA, 20 bp, Artificial Sequence
  Synthetic polynucleotide
cttgagcacgagcttggtag

SEQ ID NO: 18 - DNA, 18 bp, Artificial Sequence
  Synthetic polynucleotide
gggaaaactgcaggaaaa

SEQ ID NO: 19 - DNA, 21 bp, Artificial Sequence
  Synthetic polynucleotide
ctggacagttccctgctgtgt

SEQ ID NO: 20 - DNA, 20 bp, Artificial Sequence
  Synthetic polynucleotide
acccatcactggactggtgt

SEQ ID NO: 21 - DNA, 20 bp, Artificial Sequence
  Synthetic polynucleotide
cacatcctcaaagagcctga

SEQ ID NO: 22 - DNA, 20 bp, Artificial Sequence
  Synthetic polynucleotide
tggaaatcaagtggcaaaaa

SEQ ID NO: 23 - DNA, 18 bp, Artificial Sequence
  Synthetic polynucleotide
ctgcatgtggacgtggac

SEQ ID NO: 24 - DNA, 20 bp, Artificial Sequence
  Synthetic polynucleotide
gcgttcacctcttttccaag

SEQ ID NO: 25 - DNA, 20 bp, Artificial Sequence
  Synthetic polynucleotide
gccatgtggatttctcgttt

SEQ ID NO: 26 - DNA, 20 bp, Artificial Sequence
  Synthetic polynucleotide
aagaaaaagcctcgaaagtg

SEQ ID NO: 27 - DNA, 20 bp, Artificial Sequence
  Synthetic polynucleotide
agagcacactccagacagaa

SEQ ID NO: 28 - DNA, 20 bp, Artificial Sequence
  Synthetic polynucleotide
tgcaacgtgtatatcatcct

SEQ ID NO: 29 - DNA, 20 bp, Artificial Sequence
  Synthetic polynucleotide
acaccagagtcctttgagac

SEQ ID NO: 30 - DNA, 28 bp, Artificial Sequence
  Synthetic polynucleotide
ggagtctgtggcaactgtggagagaatg

SEQ ID NO: 31 - DNA, 31 bp, Artificial Sequence
  Synthetic polynucleotide
ccggtcttcttcattctcaatgggatccact

SEQ ID NO: 32 - DNA, 20 bp, Artificial Sequence
  Synthetic polynucleotide
gaatgtggacacggtaaaga

SEQ ID NO: 33 - DNA, 20 bp, Artificial Sequence
  Synthetic polynucleotide
taggtttgactgccaatgac

SEQ ID NO: 34 - DNA, 20 bp, Artificial Sequence
  Synthetic polynucleotide
tgggcattttctcattagcc

SEQ ID NO: 35 - DNA, 20 bp, Artificial Sequence
  Synthetic polynucleotide
ctggagcagagatgaccaca

SEQ ID NO: 36 - DNA, 18 bp, Artificial Sequence
  Synthetic polynucleotide
gacaccctcggacagcac

SEQ ID NO: 37 - DNA, 19 bp, Artificial Sequence
  Synthetic polynucleotide
gtacgggttccgctcaaag

SEQ ID NO: 38 - DNA, 20 bp, Artificial Sequence
  Synthetic polynucleotide
ctcagcgaggaagaataccg

SEQ ID NO: 39 - DNA, 20 bp, Artificial Sequence
  Synthetic polynucleotide
agtctctcaccgggcctaga

SEQ ID NO: 40 - DNA, 18 bp, Artificial Sequence
  Synthetic polynucleotide
ctgacgtgcaagggagct

SEQ ID NO: 41 - DNA, 19 bp, Artificial Sequence
  Synthetic polynucleotide
caggtttgcctagacagcg

SEQ ID NO: 42 - protein, 1082 aa, Artificial Sequence
  Synthetic polypeptide
MAPKKKRKVGIHGVPAAKRNYILGLDIGITSVGYGIIDYETRDVIDAGVRLFKEANVENNEGRRSKRGARRLKRRRRHRIQRVKKLLFDYNLLTDHSELSGINPYEARVKGLSQKLSEEEFSAALLHLAKRRGVHNVNEVEEDTGNELSTKEQISRNSKALEEKYVAELQLERLKKDGEVRGSINRFKTSDYVKEAKQLLKVQKAYHQLDQSFIDTYIDLLETRRTYYEGPGEGSPFGWKDIKEWYEMLMGHCTYFPEELRSVKYAYNADLYNALNDLNNLVITRDENEKLEYYEKFQIIENVFKQKKKPTLKQIAKEILVNEEDIKGYRVTSTGKPEFTNLKVYHDIKDITARKEIIENAELLDQIAKILTIYQSSEDIQEELTNLNSELTQEEIEQISNLKGYTGTHNLSLKAINLILDELWHTNDNQIAIFNRLKLVPKKVDLSQQKEIPTTLVDDFILSPVVKRSFIQSIKVINAIIKKYGLPNDIIIELAREKNSKDAQKMINEMQKRNRQTNERIEEIIRTTGKENAKYLIEKIKLHDMQEGKCLYSLEAIPLEDLLNNPFNYEVDHIIPRSVSFDNSFNNKVLVKQEENSKKGNRTPFQYLSSSDSKISYETFKKHILNLAKGKGRISKTKKEYLLEERDINRFSVQKDFINRNLVDTRYATRGLMNLLRSYFRVNNLDVKVKSINGGFTSFLRRKWKFKKERNKGYKHHAEDALIIANADFIFKEWKKLDKAKKVMENQMFEEKQAESMPEIETEQEYKEIFITPHQIKHIKDFKDYKYSHRVDKKPNRELINDTLYSTRKDDKGNTLIVNNLNGLYDKDNDKLKKLINKSPEKLLMYHHDPQTYQKLKLIMEQYGDEKNPLYKYYEETGNYLTKYSKKDNGPVIKKIKYYGNKLNAHLDITDDYPNSRNKVVKLSLKPYRFDVYLDNGVYKFVTVKNLDVIKKENYYEVNSKCYEEAKKLKKISNQAEFIASFYNNDLIKINGELYRVIGVNNDLLNRIEVNMIDITYREYLENMNDKRPPRIIKTIASKTQSIKKYSTDILGNLYEVKSKKHPQIIKKGKRPAATKKAGQAK

SEQ ID NO: 43 - protein, 1158 aa, Artificial Sequence
  Synthetic polypeptide
MAPKKKRKVGIHGVPAAKRNYILGLAIGITSVGYGIIDYETRDVIDAGVRLFKEANVENNEGRRSKRGARRLKRRRRHRIQRVKKLLFDYNLLTDHSELSGINPYEARVKGLSQKLSEEEFSAALLHLAKRRGVHNVNEVEEDTGNELSTKEQISRNSKALEEKYVAELQLERLKKDGEVRGSINRFKTSDYVKEAKQLLKVQKAYHQLDQSFIDTYIDLLETRRTYYEGPGEGSPFGWKDIKEWYEMLMGHCTYFPEELRSVKYAYNADLYNALNDLNNLVITRDENEKLEYYEKFQIIENVFKQKKKPTLKQIAKEILVNEEDIKGYRVTSTGKPEFTNLKVYHDIKDITARKEIIENAELLDQIAKILTIYQSSEDIQEELTNLNSELTQEEIEQISNLKGYTGTHNLSLKAINLILDELWHTNDNQIAIFNRLKLVPKKVDLSQQKEIPTTLVDDFILSPVVKRSFIQSIKVINAIIKKYGLPNDIIIELAREKNSKDAQKMINEMQKRNRQTNERIEEIIRTTGKENAKYLIEKIKLHDMQEGKCLYSLEAIPLEDLLNNPFNYEVDHIIPRSVSFDNSFNNKVLVKQEEASKKGNRTPFQYLSSSDSKISYETFKKHILNLAKGKGRISKTKKEYLLEERDINRFSVQKDFINRNLVDTRYATRGLMNLLRSYFRVNNLDVKVKSINGGFTSFLRRKWKFKKERNKGYKHHAEDALIIANADFIFKEWKKLDKAKKVMENQMFEEKQAESMPEIETEQEYKEIFITPHQIKHIKDFKDYKYSHRVDKKPNRELINDTLYSTRKDDKGNTLIVNNLNGLYDKDNDKLKKLINKSPEKLLMYHHDPQTYQKLKLIMEQYGDEKNPLYKYYEETGNYLTKYSKKDNGPVIKKIKYYGNKLNAHLDITDDYPNSRNKVVKLSLKPYRFDVYLDNGVYKFVTVKNLDVIKKENYYEVNSKCYEEAKKLKKISNQAEFIASFYNNDLIKINGELYRVIGVNNDLLNRIEVNMIDITYREYLENMNDKRPPRIIKTIASKTQSIKKYSTDILGNLYEVKSKKHPQIIKKGKRPAATKKAGQAKKKKGSDAKSLTAWSRTLVTFKDVFVDFTREEWKLLDTAQQIVYRNVMLENYKNLVSLGYQLTKPDVILRLEKGEEP

SEQ ID NO: 44 - protein, 1483 aa, Artificial Sequence
  Synthetic polypeptide
MDKKYSIGLAIGTNSVGWAVITDEYKVPSKKFKVLGNTDRHSIKKNLIGALLFDSGETAEATRLKRTARRRYTRRKNRICYLQEIFSNEMAKVDDSFFHRLEESFLVEEDKKHERHPIFGNIVDEVAYHEKYPTIYHLRKKLVDSTDKADLRLIYLALAHMIKFRGHFLIEGDLNPDNSDVDKLFIQLVQTYNQLFEENPINASGVDAKAILSARLSKSRRLENLIAQLPGEKKNGLFGNLIALSLGLTPNFKSNFDLAEDAKLQLSKDTYDDDLDNLLAQIGDQYADLFLAAKNLSDAILLSDILRVNTEITKAPLSASMIKRYDEHHQDLTLLKALVRQQLPEKYKEIFFDQSKNGYAGYIDGGASQEEFYKFIKPILEKMDGTEELLVKLNREDLLRKQRTFDNGSIPHQIHLGELHAILRRQEDFYPFLKDNREKIEKILTFRIPYYVGPLARGNSRFAWMTRKSEETITPWNFEEVVDKGASAQSFIERMTNFDKNLPNEKVLPKHSLLYEYFTVYNELTKVKYVTEGMRKPAFLSGEQKKAIVDLLFKTNRKVTVKQLKEDYFKKIECFDSVEISGVEDRFNASLGTYHDLLKIIKDKDFLDNEENEDILEDIVLTLTLFEDREMIEERLKTYAHLFDDKVMKQLKRRRYTGWGRLSRKLINGIRDKQSGKTILDFLKSDGFANRNFMQLIHDDSLTFKEDIQKAQVSGQGDSLHEHIANLAGSPAIKKGILQTVKVVDELVKVMGRHKPENIVIEMARENQTTQKGQKNSRERMKRIEEGIKELGSQILKEHPVENTQLQNEKLYLYYLQNGRDMYVDQELDINRLSDYDVDAIVPQSFLKDDSIDNKVLTRSDKNRGKSDNVPSEEVVKKMKNYWRQLLNAKLITQRKFDNLTKAERGGLSELDKAGFIKRQLVETRQITKHVAQILDSRMNTKYDENDKLIREVKVITLKSKLVSDFRKDFQFYKVREINNYHHAHDAYLNAVVGTALIKKYPKLESEFVYGDYKVYDVRKMIAKSEQEIGKATAKYFFYSNIMNFFKTEITLANGEIRKRPLIETNGETGEIVWDKGRDFATVRKVLSMPQVNIVKKTEVQTGGFSKESILPKRNSDKLIARKKDWDPKKYGGFDSPTVAYSVLVVAKVEKGKSKKLKSVKELLGITIMERSSFEKNPIDFLEAKGYKEVKKDLIIKLPKYSLFELENGRKRMLASAGELQKGNELALPSKYVNFLYLASHYEKLKGSPEDNEQKQLFVEQHKHYLDEIIEQISEFSKRVILADANLDKVLSAYNKHRDKPIREQAENIIHLFTLTNLGAPAAFKYFDTTIDRKRYTSTKEVLDATLIHQSITGLYETRIDLSQLGGDGTGGPKKKRKVYPYDVPDYAGYPYDVPDYAGSYPYDVPDYAGSMDAKSLTAWSRTLVTFKDVFVDFTREEWKLLDTAQQIVYRNVMLENYKNLVSLGYQLTKPDVILRLEKGEEP

SEQ ID NO: 45 - protein, 1069 aa, Artificial Sequence
  Synthetic polypeptide
MAPKKKRKVGIHGVPAAKRNYILGLAIGITSVGYGIIDYETRDVIDAGVRLFKEANVENNEGRRSKRGARRLKRRRRHRIQRVKKLLFDYNLLTDHSELSGINPYEARVKGLSQKLSEEEFSAALLHLAKRRGVHNVNEVEEDTGNELSTKEQISRNSKALEEKYVAELQLERLKKDGEVRGSINRFKTSDYVKEAKQLLKVQKAYHQLDQSFIDTYIDLLETRRTYYEGPGEGSPFGWKDIKEWYEMLMGHCTYFPEELRSVKYAYNADLYNALNDLNNLVITRDENEKLEYYEKFQIIENVFKQKKKPTLKQIAKEILVNEEDIKGYRVTSTGKPEFTNLKVYHDIKDITARKEIIENAELLDQIAKILTIYQSSEDIQEELTNLNSELTQEEIEQISNLKGYTGTHNLSLKAINLILDELWHTNDNQIAIFNRLKLVPKKVDLSQQKEIPTTLVDDFILSPVVKRSFIQSIKVINAIIKKYGLPNDIIIELAREKNSKDAQKMINEMQKRNRQTNERIEEIIRTTGKENAKYLIEKIKLHDMQEGKCLYSLEAIPLEDLLNNPFNYEVDHIIPRSVSFDNSFNNKVLVKQEEASKKGNRTPFQYLSSSDSKISYETFKKHILNLAKGKGRISKTKKEYLLEERDINRFSVQKDFINRNLVDTRYATRGLMNLLRSYFRVNNLDVKVKSINGGFTSFLRRKWKFKKERNKGYKHHAEDALIIANADFIFKEWKKLDKAKKVMENQMFEEKQAESMPEIETEQEYKEIFITPHQIKHIKDFKDYKYSHRVDKKPNRELINDTLYSTRKDDKGNTLIVNNLNGLYDKDNDKLKKLINKSPEKLLMYHHDPQTYQKLKLIMEQYGDEKNPLYKYYEETGNYLTKYSKKDNGPVIKKIKYYGNKLNAHLDITDDYPNSRNKVVKLSLKPYRFDVYLDNGVYKFVTVKNLDVIKKENYYEVNSKCYEEAKKLKKISNQAEFIASFYNNDLIKINGELYRVIGVNNDLLNRIEVNMIDITYREYLENMNDKRPPRIIKTIASKTQSIKKYSTDILGNLYEVKSKKHPQIIKKG